European Patent Application EP 4 151 083 A1, published March 22, 2023. Title: HIGH-REBAUDIOSIDE E-CONTENT STEVIA PLANT. Applicant: SUNTORY HOLDINGS LIMITED. The sequence listing filed with the application follows.

SEQUENCE LISTING (93 sequences)

SEQ ID NO: 1 - DNA, 203 bp, Stevia rebaudiana
aattatatgatagaaattgttttcacattttgtgtgccatacacgtcaacgcctctaagccacacgattaaggtatgacatttagaataaaatcttttattattggaagatagagacaaaatcttttctttccttatttattttttataataattacacgcatcttctattctcaactactttaacctatatgcgctagtcca

SEQ ID NO: 2 - DNA, 364 bp, Stevia rebaudiana
gaaactgaaagagaagtaagataacagaatgcgtttyttcgtaaataatcttttcttttatttttatcttcaaaaaataaataaccaagatttgtttggatttgtttctatttatttagacaaatcattattaatatttaatmtttcyccgtgaattatatgatagaaattgttttcacattttgtgtgccayacacgtcaacgcctctaagccacacgattaaggtatgacatttagaataaaatcttttattattggaagatagagacaaaatcttttctttccttatttattttttataataattacacgcatcttctattctcaactactttaacctatatgcgctagtccactacgtag

SEQ ID NO: 3 - DNA, 202 bp, Stevia rebaudiana
agagaagtaagwtaacagaatgcgtttcttcgtaaataatcttttcttttatttttatcttcaaaaaataaataaccaagatttgtttggatttgtttctatttatttagacaaatcattattaatatttaatmtttcyccgtgaattatatgatagaaattgttttcacattttgtgtgccayacacgtcaacgcctctaa

SEQ ID NO: 4 - DNA, 137 bp, Stevia rebaudiana
ccaagatttgtttggatttgtttctatttatttagacaaatcattattaatatttaatatttcyccgtgaattatatgatagaaattgttttcacattttgtgtgccayacacgtcaacgcctctaagccacacgat

SEQ ID NO: 5 - DNA, 137 bp, Stevia rebaudiana
ccaagatttgtttggatttgtttctatttatttagacaaatcattattaatatttaatmtttccccgtgaattatatgatagaaattgttttcacattttgtgtgccayacacgtcaacgcctctaagccacacgat

SEQ ID NO: 6 - DNA, 39 bp, Artificial Sequence
  Synthetic DNA
aattatatgatagaaattgttttcacattttgtgtgcca

SEQ ID NO: 7 - DNA, 26 bp, Artificial Sequence
  Synthetic DNA
tggactagcgcatataggttaaagta

SEQ ID NO: 8 - DNA, 20 bp, Artificial Sequence
  Synthetic DNA
gaaactgaaagagaagtaag

SEQ ID NO: 9 - DNA, 20 bp, Artificial Sequence
  Synthetic DNA
ctacgtagtggactagcgca

SEQ ID NO: 10 - DNA, 24 bp, Artificial Sequence
  Synthetic DNA
agagaagtaagwtaacagaatgcg

SEQ ID NO: 11 - DNA, 20 bp, Artificial Sequence
  Synthetic DNA
ttagaggcgttgacgtgtrt

SEQ ID NO: 12 - DNA, 25 bp, Artificial Sequence
  Synthetic DNA
ccaagatttgtttggatttgtttct

SEQ ID NO: 13 - DNA, 19 bp, Artificial Sequence
  Synthetic DNA
atcgtgtggcttagaggcg

SEQ ID NO: 14 - DNA, 25 bp, Artificial Sequence
  Synthetic DNA
ccaagatttgtttggatttgtttct

SEQ ID NO: 15 - DNA, 19 bp, Artificial Sequence
  Synthetic DNA
atcgtgtggcttagaggcg

SEQ ID NO: 16 - DNA, 203 bp, Stevia rebaudiana
aattatatgatagaaattgttttcacattttgtgtgccacacacgtcaacgcctctaagccacacgattaaggtatgacatttagaataaaatcttttattattggaagatagagacaaaatcttttctttccttatttattttttataataattacacgcatcttctattctcaactactttaacctatatgcgctagtcca

SEQ ID NO: 17 - DNA, 21 bp, Stevia rebaudiana
ttgtgtgccacacacgtcaac

SEQ ID NO: 18 - DNA, 41 bp, Stevia rebaudiana
ttttcacattttgtgtgccacacacgtcaacgcctctaagc

SEQ ID NO: 19 - DNA, 61 bp, Stevia rebaudiana
atagaaattgttttcacattttgtgtgccacacacgtcaacgcctctaagccacacgatta

SEQ ID NO: 20 - DNA, 364 bp, Stevia rebaudiana
gaaactgaaagagaagtaagttaacagaatgcgtttyttcgtaaataatcttttcttttatttttatcttcaaaaaataaataaccaagatttgtttggatttgtttctatttatttagacaaatcattattaatatttaatmtttcyccgtgaattatatgatagaaattgttttcacattttgtgtgccayacacgtcaacgcctctaagccacacgattaaggtatgacatttagaataaaatcttttattattggaagatagagacaaaatcttttctttccttatttattttttataataattacacgcatcttctattctcaactactttaacctatatgcgctagtccactacgtag

SEQ ID NO: 21 - DNA, 21 bp, Stevia rebaudiana
gagaagtaagttaacagaatg

SEQ ID NO: 22 - DNA, 41 bp, Stevia rebaudiana
gaaactgaaagagaagtaagttaacagaatgcgtttyttcg

SEQ ID NO: 23 - DNA, 61 bp, Stevia rebaudiana
aatgtttaaggaaactgaaagagaagtaagttaacagaatgcgtttyttcgtaaataatct

SEQ ID NO: 24 - DNA, 202 bp, Stevia rebaudiana
agagaagtaagwtaacagaatgcgttttttcgtaaataatcttttcttttatttttatcttcaaaaaataaataaccaagatttgtttggatttgtttctatttatttagacaaatcattattaatatttaatmtttcyccgtgaattatatgatagaaattgttttcacattttgtgtgccayacacgtcaacgcctctaa

SEQ ID NO: 25 - DNA, 21 bp, Stevia rebaudiana
gaatgcgttttttcgtaaata

SEQ ID NO: 26 - DNA, 41 bp, Stevia rebaudiana
taagwtaacagaatgcgttttttcgtaaataatcttttctt

SEQ ID NO: 27 - DNA, 61 bp, Stevia rebaudiana
gaaagagaagtaagwtaacagaatgcgttttttcgtaaataatcttttcttttatttttat

SEQ ID NO: 28 - DNA, 137 bp, Stevia rebaudiana
ccaagatttgtttggatttgtttctatttatttagacaaatcattattaatatttaatctttcyccgtgaattatatgatagaaattgttttcacattttgtgtgccayacacgtcaacgcctctaagccacacgat

SEQ ID NO: 29 - DNA, 21 bp, Stevia rebaudiana
aatatttaatctttcyccgtg

SEQ ID NO: 30 - DNA, 41 bp, Stevia rebaudiana
aatcattattaatatttaatctttcyccgtgaattatatga

SEQ ID NO: 31 - DNA, 61 bp, Stevia rebaudiana
tatttagacaaatcattattaatatttaatctttcyccgtgaattatatgatagaaattgt

SEQ ID NO: 32 - DNA, 137 bp, Stevia rebaudiana
ccaagatttgtttggatttgtttctatttatttagacaaatcattattaatatttaatmtttctccgtgaattatatgatagaaattgttttcacattttgtgtgccayacacgtcaacgcctctaagccacacgat

SEQ ID NO: 33 - DNA, 21 bp, Stevia rebaudiana
ttaatmtttctccgtgaatta

SEQ ID NO: 34 - DNA, 41 bp, Stevia rebaudiana
ttattaatatttaatmtttctccgtgaattatatgatagaa

SEQ ID NO: 35 - DNA, 61 bp, Stevia rebaudiana
agacaaatcattattaatatttaatmtttctccgtgaattatatgatagaaattgttttca

SEQ ID NO: 36 - DNA, 39 bp, Artificial Sequence
  Synthetic DNA
aattatatgatagaaattgttttcacattttgtgtgccg

SEQ ID NO: 37 - DNA, 26 bp, Artificial Sequence
  Synthetic DNA
tggactagcgcatataggttaaagta

SEQ ID NO: 38 - DNA, 203 bp, Artificial Sequence
  Synthetic DNA
aattatatgatagaaattgttttcacattttgtgtgccgcacacgtcaacgcctctaagccacacgattaaggtatgacatttagaataaaatcttttattattggaagatagagacaaaatcttttctttccttatttattttttataataattacacgcatcttctattctcaactactttaacctatatgcgctagtcca

SEQ ID NO: 39 - DNA, 203 bp, Artificial Sequence
  Synthetic DNA
aattatatgatagaaattgttttcacattttgtgtgccgtacacgtcaacgcctctaagccacacgattaaggtatgacatttagaataaaatcttttattattggaagatagagacaaaatcttttctttccttatttattttttataataattacacgcatcttctattctcaactactttaacctatatgcgctagtcca

SEQ ID NO: 40 - DNA, 40 bp, Artificial Sequence
  Synthetic DNA
aattatatgatagaaattgttttcacattttgtgtgccgt

SEQ ID NO: 41 - DNA, 163 bp, Artificial Sequence
  Synthetic DNA
acacgtcaacgcctctaagccacacgattaaggtatgacatttagaataaaatcttttattattggaagatagagacaaaatcttttctttccttatttattttttataataattacacgcatcttctattctcaactactttaacctatatgcgctagtcca

SEQ ID NO: 42 - DNA, 20 bp, Artificial Sequence
  Synthetic DNA
gaaactgaaagagaagaacg

SEQ ID NO: 43 - DNA, 20 bp, Artificial Sequence
  Synthetic DNA
ctacgtagtggactagcgca

SEQ ID NO: 44 - DNA, 364 bp, Artificial Sequence
  Synthetic DNA
gaaactgaaagagaagaacgttaacagaatgcgtttyttcgtaaataatcttttcttttatttttatcttcaaaaaataaataaccaagatttgtttggatttgtttctatttatttagacaaatcattattaatatttaatmtttcyccgtgaattatatgatagaaattgttttcacattttgtgtgccayacacgtcaacgcctctaagccacacgattaaggtatgacatttagaataaaatcttttattattggaagatagagacaaaatcttttctttccttatttattttttataataattacacgcatcttctattctcaactactttaacctatatgcgctagtccactacgtag

SEQ ID NO: 45 - DNA, 364 bp, Artificial Sequence
  Synthetic DNA
gaaactgaaagagaagaacgataacagaatgcgtttyttcgtaaataatcttttcttttatttttatcttcaaaaaataaataaccaagatttgtttggatttgtttctatttatttagacaaatcattattaatatttaatmtttcyccgtgaattatatgatagaaattgttttcacattttgtgtgccayacacgtcaacgcctctaagccacacgattaaggtatgacatttagaataaaatcttttattattggaagatagagacaaaatcttttctttccttatttattttttataataattacacgcatcttctattctcaactactttaacctatatgcgctagtccactacgtag

SEQ ID NO: 46 - DNA, 18 bp, Artificial Sequence
  Synthetic DNA
gaaactgaaagagaagaa

SEQ ID NO: 47 - DNA, 346 bp, Artificial Sequence
  Synthetic DNA
cgttaacagaatgcgtttyttcgtaaataatcttttcttttatttttatcttcaaaaaataaataaccaagatttgtttggatttgtttctatttatttagacaaatcattattaatatttaatmtttcyccgtgaattatatgatagaaattgttttcacattttgtgtgccayacacgtcaacgcctctaagccacacgattaaggtatgacatttagaataaaatcttttattattggaagatagagacaaaatcttttctttccttatttattttttataataattacacgcatcttctattctcaactactttaacctatatgcgctagtccactacgtag

SEQ ID NO: 48 - DNA, 20 bp, Artificial Sequence
  Synthetic DNA
taagwtaacagaatgcgagc

SEQ ID NO: 49 - DNA, 20 bp, Artificial Sequence
  Synthetic DNA
acgtagtggactagcgcata

SEQ ID NO: 50 - DNA, 353 bp, Artificial Sequence
  Synthetic DNA
taagwtaacagaatgcgagctttcgtaaataatcttttcttttatttttatcttcaaaaaataaataaccaagatttgtttggatttgtttctatttatttagacaaatcattattaatatttaatmtttcyccgtgaattatatgatagaaattgttttcacattttgtgtgccayacacgtcaacgcctctaagccacacgattaaggtatgacatttagaataaaatcttttattattggaagatagagacaaaatcttttctttccttatttattttttataataattacacgcatcttctattctcaactactttaacctatatgcgctatgcgctagtccactacgt

SEQ ID NO: 51 - DNA, 353 bp, Artificial Sequence
  Synthetic DNA
taagwtaacagaatgcgagccttcgtaaataatcttttcttttatttttatcttcaaaaaataaataaccaagatttgtttggatttgtttctatttatttagacaaatcattattaatatttaatmtttcyccgtgaattatatgatagaaattgttttcacattttgtgtgccayacacgtcaacgcctctaagccacacgattaaggtatgacatttagaataaaatcttttattattggaagatagagacaaaatcttttctttccttatttattttttataataattacacgcatcttctattctcaactactttaacctatatgcgctatgcgctagtccactacgt

SEQ ID NO: 52 - DNA, 19 bp, Artificial Sequence
  Synthetic DNA
taagwtaacagaatgcgag

SEQ ID NO: 53 - DNA, 334 bp, Artificial Sequence
  Synthetic DNA
ctttcgtaaataatcttttcttttatttttatcttcaaaaaataaataaccaagatttgtttggatttgtttctatttatttagacaaatcattattaatatttaatmtttcyccgtgaattatatgatagaaattgttttcacattttgtgtgccayacacgtcaacgcctctaagccacacgattaaggtatgacatttagaataaaatcttttattattggaagatagagacaaaatcttttctttccttatttattttttataataattacacgcatcttctattctcaactactttaacctatatgcgctatgcgctagtccactacgt

SEQ ID NO: 54 - DNA, 21 bp, Artificial Sequence
  Synthetic DNA
aaatcattattaatatttaag

SEQ ID NO: 55 - DNA, 20 bp, Artificial Sequence
  Synthetic DNA
tggcgccggcgaacggttgt

SEQ ID NO: 56 - DNA, 349 bp, Artificial Sequence
  Synthetic DNA
aaatcattattaatatttaagctttcyccgtgaattatatgatagaaattgttttcacattttgtgtgccayacacgtcaacgcctctaagccacacgattaaggtatgacatttagaataaaatcttttattattggaagatagagacaaaatcttttctttccttatttattttttataataattacacgcatcttctattctcaactactttaacctatatgcgctagtccactacgtagagtcgttcattctgttttcgagtttctacgttcattctgtttttgagtgtaaacatcagtcaaatcccatggaaaataaaacggagacaaccgttcgccggcgcca

SEQ ID NO: 57 - DNA, 349 bp, Artificial Sequence
  Synthetic DNA
aaatcattattaatatttaagatttcyccgtgaattatatgatagaaattgttttcacattttgtgtgccayacacgtcaacgcctctaagccacacgattaaggtatgacatttagaataaaatcttttattattggaagatagagacaaaatcttttctttccttatttattttttataataattacacgcatcttctattctcaactactttaacctatatgcgctagtccactacgtagagtcgttcattctgttttcgagtttctacgttcattctgtttttgagtgtaaacatcagtcaaatcccatggaaaataaaacggagacaaccgttcgccggcgcca

SEQ ID NO: 58 - DNA, 21 bp, Artificial Sequence
  Synthetic DNA
aaatcattattaatatttaag

SEQ ID NO: 59 - DNA, 328 bp, Artificial Sequence
  Synthetic DNA
ctttcyccgtgaattatatgatagaaattgttttcacattttgtgtgccayacacgtcaacgcctctaagccacacgattaaggtatgacatttagaataaaatcttttattattggaagatagagacaaaatcttttctttccttatttattttttataataattacacgcatcttctattctcaactactttaacctatatgcgctagtccactacgtagagtcgttcattctgttttcgagtttctacgttcattctgtttttgagtgtaaacatcagtcaaatcccatggaaaataaaacggagacaaccgttcgccggcgcca

SEQ ID NO: 60 - DNA, 22 bp, Artificial Sequence
  Synthetic DNA
cattattaatatttaatmtagc

SEQ ID NO: 61 - DNA, 20 bp, Artificial Sequence
  Synthetic DNA
tctctggcgccggcgaacgg

SEQ ID NO: 62 - DNA, 349 bp, Artificial Sequence
  Synthetic DNA
cattattaatatttaatmtagctccgtgaattatatgatagaaattgttttcacattttgtgtgccayacacgtcaacgcctctaagccacacgattaaggtatgacatttagaataaaatcttttattattggaagatagagacaaaatcttttctttccttatttattttttataataattacacgcatcttctattctcaactactttaacctatatgcgctagtccactacgtagagtcgttcattctgttttcgagtttctacgttcattctgtttttgagtgtaaacatcagtcaaatcccatggaaaataaaacggagacaaccgttcgccggcgccagaga

SEQ ID NO: 63 - DNA, 349 bp, Artificial Sequence
  Synthetic DNA
cattattaatatttaatmtagccccgtgaattatatgatagaaattgttttcacattttgtgtgccayacacgtcaacgcctctaagccacacgattaaggtatgacatttagaataaaatcttttattattggaagatagagacaaaatcttttctttccttatttattttttataataattacacgcatcttctattctcaactactttaacctatatgcgctagtccactacgtagagtcgttcattctgttttcgagtttctacgttcattctgtttttgagtgtaaacatcagtcaaatcccatggaaaataaaacggagacaaccgttcgccggcgccagaga

SEQ ID NO: 64 - DNA, 21 bp, Artificial Sequence
  Synthetic DNA
cattattaatatttaatmtag

SEQ ID NO: 65 - DNA, 328 bp, Artificial Sequence
  Synthetic DNA
ctccgtgaattatatgatagaaattgttttcacattttgtgtgccayacacgtcaacgcctctaagccacacgattaaggtatgacatttagaataaaatcttttattattggaagatagagacaaaatcttttctttccttatttattttttataataattacacgcatcttctattctcaactactttaacctatatgcgctagtccactacgtagagtcgttcattctgttttcgagtttctacgttcattctgtttttgagtgtaaacatcagtcaaatcccatggaaaataaaacggagacaaccgttcgccggcgccagaga

SEQ ID NO: 66 - DNA, 21 bp, Stevia rebaudiana
ttgtgtgccatacacgtcaac

SEQ ID NO: 67 - DNA, 41 bp, Stevia rebaudiana
ttttcacattttgtgtgccatacacgtcaacgcctctaagc

SEQ ID NO: 68 - DNA, 61 bp, Stevia rebaudiana
atagaaattgttttcacattttgtgtgccatacacgtcaacgcctctaagccacacgatta

SEQ ID NO: 69 - DNA, 21 bp, Stevia rebaudiana
gagaagtaagataacagaatg

SEQ ID NO: 70 - DNA, 41 bp, Stevia rebaudiana
gaaactgaaagagaagtaagataacagaatgcgtttyttcg

SEQ ID NO: 71 - DNA, 61 bp, Stevia rebaudiana
aatgtttaaggaaactgaaagagaagtaagataacagaatgcgtttyttcgtaaataatct

SEQ ID NO: 72 - DNA, 21 bp, Stevia rebaudiana
gaatgcgtttcttcgtaaata

SEQ ID NO: 73 - DNA, 41 bp, Stevia rebaudiana
taagwtaacagaatgcgtttcttcgtaaataatcttttctt

SEQ ID NO: 74 - DNA, 61 bp, Stevia rebaudiana
gaaagagaagtaagwtaacagaatgcgtttcttcgtaaataatcttttcttttatttttat

SEQ ID NO: 75 - DNA, 21 bp, Stevia rebaudiana
aatatttaatatttcyccgtg

SEQ ID NO: 76 - DNA, 41 bp, Stevia rebaudiana
aatcattattaatatttaatatttcyccgtgaattatatga

SEQ ID NO: 77 - DNA, 61 bp, Stevia rebaudiana
tatttagacaaatcattattaatatttaatatttcyccgtgaattatatgatagaaattgt

SEQ ID NO: 78 - DNA, 21 bp, Stevia rebaudiana
ttaatmtttccccgtgaatta

SEQ ID NO: 79 - DNA, 41 bp, Stevia rebaudiana
ttattaatatttaatmtttccccgtgaattatatgatagaa

SEQ ID NO: 80 - DNA, 61 bp, Stevia rebaudiana
agacaaatcattattaatatttaatmtttccccgtgaattatatgatagaaattgttttca

SEQ ID NO: 81 - DNA, 20 bp, Artificial Sequence
  Synthetic DNA
ttttcacattttgtgtgtca

SEQ ID NO: 82 - DNA, 20 bp, Artificial Sequence
  Synthetic DNA
ttttcacattttgtgtgccg

SEQ ID NO: 83 - DNA, 340 bp, Artificial Sequence
  Synthetic DNA
ttttcacattttgtgtgccatacacgtcaacgcctctaagccacacgattaaggtatgacatttagaataaaatcttttattattggaagatagagacaaaatcttttctttccttatttattttttataataattacacgcatcttctattctcaactactttaacctatatgcgctagtccactacgtagagtcgttcattctgttttcgagtttctacgttcattctgtttttgagtgtaaacatcagtcaaatcccatggaaaataaaacggagacaaccgttcgccggcgccagagaataatattgttcccggtaccatttcaaggccacataag

SEQ ID NO: 84 - DNA, 340 bp, Artificial Sequence
  Synthetic DNA
ttttcacattttgtgtgccacacacgtcaacgcctctaagccacacgattaaggtatgacatttagaataaaatcttttattattggaagatagagacaaaatcttttctttccttatttattttttataataattacacgcatcttctattctcaactactttaacctatatgcgctagtccactacgtagagtcgttcattctgttttcgagtttctacgttcattctgtttttgagtgtaaacatcagtcaaatcccatggaaaataaaacggagacaaccgttcgccggcgccagagaataatattgttcccggtaccatttcaaggccacataag

SEQ ID NO: 85 - DNA, 21 bp, Artificial Sequence
  Synthetic DNA
cttatgtggccttgaaatggt

SEQ ID NO: 86 - DNA, 20 bp, Artificial Sequence
  Synthetic DNA
gaaactgaaagagaagtagc

SEQ ID NO: 87 - DNA, 20 bp, Artificial Sequence
  Synthetic DNA
gaaactgaaagagaagttaa

SEQ ID NO: 88 - DNA, 20 bp, Artificial Sequence
  Synthetic DNA
taagwtaacagaatgagatc

SEQ ID NO: 89 - DNA, 20 bp, Artificial Sequence
  Synthetic DNA
taagwtaacagaatgagtac

SEQ ID NO: 90 - DNA, 21 bp, Artificial Sequence
  Synthetic DNA
aaatcattattaatatttgat

SEQ ID NO: 91 - DNA, 21 bp, Artificial Sequence
  Synthetic DNA
aaatcattattaatattagat

SEQ ID NO: 92 - DNA, 22 bp, Artificial Sequence
  Synthetic DNA
cattattaatatttaatmttga

SEQ ID NO: 93 - DNA, 22 bp, Artificial Sequence
  Synthetic DNA
cattattaatatttaatmgatc